European Patent Specification EP 3 708 671 B1, published April 2, 2025. Title: METHODS AND COMPOSITIONS FOR MODIFYING A TARGETED LOCUS. Applicant: Auerbach, Wojtek Frendewey, David Droguett, Gustavo Gagliardi, Anthony Kuno, Junko Valenzuela , David M. The sequence listing filed with the application follows.

SEQUENCE LISTING (20 sequences)

SEQ ID NO: 1 - DNA, 23 bp, Artificial Sequence
  a target locus that is linked to a guide RNA (gRNA)
  misc_feature 2, 3, 4, 5, 6, 7, 8, 9, 10, 11, 12, 13, 14, 15, 16, 17, 18,19, 20, 21: n = A,T,C or G
gnnnnnnnnnnnnnnnnnnnngg

SEQ ID NO: 2 - RNA, 80 nt, Artificial Sequence
  a guide RNA (gRNA)
guuuuagagcuagaaauagcaaguuaaaauaaggcuaguccguuaucaacuugaaaaaguggcaccgagucggugcuuuu

SEQ ID NO: 3 - RNA, 42 nt, Artificial Sequence
  a guide RNA (gRNA)
guuuuagagcuagaaauagcaaguuaaaauaaggcuaguccg

SEQ ID NO: 4 - RNA, 30 nt, Artificial Sequence
  a crRNA
guuuuagagcuagaaauagcaaguuaaaau

SEQ ID NO: 5 - RNA, 33 nt, Artificial Sequence
  a crRNA
guuuuagagcuagaaauagcaaguuaaaauaag

SEQ ID NO: 6 - RNA, 26 nt, Artificial Sequence
  a crRNA
gaguccgagcagaagaagaaguuuua

SEQ ID NO: 7 - RNA, 12 nt, Artificial Sequence
  a tracrRNA
aaggcuaguccg

SEQ ID NO: 8 - RNA, 50 nt, Artificial Sequence
  a tracrRNA
aaggcuaguccguuaucaacuugaaaaaguggcaccgagucggugcuuuu

SEQ ID NO: 9 - DNA, 40 bp, Artificial Sequence
  Neo-ZFN(1,2): NUCLEASE BINDING SITE/cut site
gggcgcccggttctttttgtcaagaccgacctgtccggtg

SEQ ID NO: 10 - DNA, 36 bp, Artificial Sequence
  ZFN(3,4): NUCLEASE BINDING SITE/cut site
ccggttctttttgtcaagaccgacctgtccggtgcc

SEQ ID NO: 11 - DNA, 42 bp, Artificial Sequence
  ZFN(1,2): NUCLEASE BINDING SITE/cut site
tgcgatcgctgcggccgatcttagccagacgagcgggttcgg

SEQ ID NO: 12 - DNA, 36 bp, Artificial Sequence
  Hyg-ZFN(3,4): NUCLEASE BINDING SITE/cut site
cgctgcggccgatcttagccagacgagcgggttcgg

SEQ ID NO: 13 - RNA, 20 nt, Artificial Sequence
  gRNA Neo Crispr#1
ugcgcaaggaacgcccgucg

SEQ ID NO: 14 - RNA, 20 nt, Artificial Sequence
  gRNA Neo Crispr#2
ggcagcgcggcuaucguggc

SEQ ID NO: 15 - RNA, 20 nt, Artificial Sequence
  gRNA Neo Crispr#3
acgaggcagcgcggcuaucg

SEQ ID NO: 16 - RNA, 20 nt, Artificial Sequence
  gRNA Neo Crispr#4
gcucugaugccgccguguuc

SEQ ID NO: 17 - RNA, 20 nt, Artificial Sequence
  gRNA Hyg Crispr#1
acgagcggguucggcccauu

SEQ ID NO: 18 - RNA, 20 nt, Artificial Sequence
  gRNA Hyg Crispr#2
cuuagccagacgagcggguu

SEQ ID NO: 19 - RNA, 20 nt, Artificial Sequence
  gRNA Hyg Crispr#3
gccgaucuuagccagacgag

SEQ ID NO: 20 - RNA, 20 nt, Artificial Sequence
  gRNA Hyg Crispr#4
cgaccugaugcagcucucgg